European Patent Specification EP 3 816 188 B1, published March 13, 2024. Title: Separating Agent. Applicant: National University Corporation Kyoto Institute of Technology Daicel Corporation. The sequence listing filed with the application follows.

SEQUENCE LISTING (33 sequences)

SEQ ID NO: 1 - protein, 119 aa, Oryctolagus cuniculus
QEQLVESGGGLVKPGGTLTLTCTVSGIDLSSYAMSWVRQVPGKGLEWIGIIGSGGGTAYANWAKGRFTISKTSSTTVDLKMTSLTTEDTATYFCATDYGIYGYAYGHLWGPGTLVTVTS

SEQ ID NO: 2 - protein, 15 aa, Artificial Sequence
  spacer
GGGGSGGGGSGGGGS

SEQ ID NO: 3 - protein, 111 aa, Oryctolagus cuniculus
ELVMTQTASPVSAAVGGTVTIKCQASQSISTALAWYQQRPGQPPKLLIYDASTLASGVSSRFKGSGSGTEFTLTISDLECADAATYYCQTYFGSDTDNAFGEGTEVEITGS

SEQ ID NO: 4 - protein, 5 aa, Artificial Sequence
  spacer
AAALE

SEQ ID NO: 5 - protein, 250 aa, Artificial Sequence
  reference
QEQLVESGGGLVKPGGTLTLTCTVSGIDLSSYAMSWVRQVPGKGLEWIGIIGSGGGTAYANWAKGRFTISKTSSTTVDLKMTSLTTEDTATYFCATDYGIYGYAYGHLWGPGTLVTVTSGGGGSGGGGSGGGGSELVMTQTASPVSAAVGGTVTIKCQASQSISTALAWYQQRPGQPPKLLIYDASTLASGVSSRFKGSGSGTEFTLTISDLECADAATYYCQTYFGSDTDNAFGEGTEVEITGSAAALE

SEQ ID NO: 6 - protein, 256 aa, Artificial Sequence
  comparative
QEQLVESGGGLVTPGGTLTLTCTVSGIDLSSYAMSWVRQVPGEGLEWIGIIGSGGGTAYANWARGRFTISRTSSTTVDLRMTSLTTEDTATYFCATDYGIYGYAYGHLWGPGTLVTVTSGGGGSGGGGSGGGGSELVMTQTASPVSAAVGGTVTINCQASQSISTALAWYQQRPGQPPRLLIYDASTLASGVSSRFSGSGSGTEFTLTISDLESADAATYYCQTYFGSDTDNAFGEGTEVEITGSAAAGGGGSKIE

SEQ ID NO: 7 - protein, 258 aa, Artificial Sequence
  example
QEQLVESGGGLVTPGGTLTLTCTVSGIDLSSYAMSWVRQVPGEGLEWIGIIGSGGGTAYANWARGRFTISRTSSTTVDLRMTSLTTEDTATYFCATDYGIYGYAYGHLWGPGTLVTVTSGGGGSGGGGSGGGGSELVMTQTASPVSAAVGGTVTINCQASQSISTALAWYQQRPGQPPRLLIYDASTLASGVSSRFSGSGSGTEFTLTISDLESADAATYYCQTYFGSDTDNAFGEGTEVEITGSAAAGGGGSKKKIE

SEQ ID NO: 8 - protein, 260 aa, Artificial Sequence
  example
QEQLVESGGGLVTPGGTLTLTCTVSGIDLSSYAMSWVRQVPGEGLEWIGIIGSGGGTAYANWARGRFTISRTSSTTVDLRMTSLTTEDTATYFCATDYGIYGYAYGHLWGPGTLVTVTSGGGGSGGGGSGGGGSELVMTQTASPVSAAVGGTVTINCQASQSISTALAWYQQRPGQPPRLLIYDASTLASGVSSRFSGSGSGTEFTLTISDLESADAATYYCQTYFGSDTDNAFGEGTEVEITGSAAAGGGGSKKKKKIE

SEQ ID NO: 9 - DNA, 750 bp, Artificial Sequence
  reference
caggagcagctggtggagtccgggggaggcctggtcaagcctggaggaaccctgacactcacctgcacagtctctggaatcgacctcagtagctatgcaatgagctgggtccgccaggttccagggaaggggctggaatggatcggaatcattggtagtggtggtggcacagcctacgcgaactgggcgaaaggccgattcaccatctccaaaacctcgtcgaccacggtggatctgaaaatgaccagtctgacaaccgaggacacggccacctatttctgtgccaccgattacggcatttatggttatgcttatggtcacttgtggggcccaggcaccctcgtcaccgtcactagtggtggaggcggttcaggcggaggtggctctggcggtggcggatccgagctcgtgatgacccagactgcatcccccgtgtctgcagctgtgggaggcacagtcaccatcaagtgccaggccagtcagagcattagcactgcattagcctggtatcagcagagaccagggcagcctcccaagctcctgatctacgatgcatccactctggcatctggggtctcatcgcggttcaaaggcagtggatctgggacagagttcactctcaccatcagcgacctggagtgtgccgatgctgccacttactactgtcaaacctattttggtagtgatactgataatgctttcggcgaagggaccgaggtggagatcacaggttcggcggccgcactcgag

SEQ ID NO: 10 - DNA, 768 bp, Artificial Sequence
  comparative
caggagcagctggtggagtccgggggaggcctggtcactcctggaggaaccctgacactcacctgcacagtctctggaatcgacctcagtagctatgcaatgagctgggtccgccaggttccaggggaagggctggaatggatcggaatcattggtagtggtggtggcacagcctacgcgaactgggcgcgtggccgattcaccatctcccgtacctcgtcgaccacggtggatctgcgtatgaccagtctgacaaccgaggacacggccacctatttctgtgccaccgattacggcatttatggttatgcttatggtcacttgtggggcccaggcaccctcgtcaccgtcactagtggtggaggcggttcaggcggaggtggctctggcggtggcggatccgagctcgtgatgacccagactgcatcccccgtgtctgcagctgtgggaggcacagtcaccatcaattgccaggccagtcagagcattagcactgcattagcctggtatcagcagagaccagggcagcctccccgtctcctgatctacgatgcatccactctggcatctggggtctcatcgcggttctctggcagtggatctgggacagagttcactctcaccatcagcgacctggagagtgccgatgctgccacttactactgtcaaacctattttggtagtgatactgataatgctttcggcgaagggaccgaggtggagatcacaggttcggcggccgcaggtggaggcggttcaaaaatcgag

SEQ ID NO: 11 - DNA, 774 bp, Artificial Sequence
  example
caggagcagctggtggagtccgggggaggcctggtcactcctggaggaaccctgacactcacctgcacagtctctggaatcgacctcagtagctatgcaatgagctgggtccgccaggttccaggggaagggctggaatggatcggaatcattggtagtggtggtggcacagcctacgcgaactgggcgcgtggccgattcaccatctcccgtacctcgtcgaccacggtggatctgcgtatgaccagtctgacaaccgaggacacggccacctatttctgtgccaccgattacggcatttatggttatgcttatggtcacttgtggggcccaggcaccctcgtcaccgtcactagtggtggaggcggttcaggcggaggtggctctggcggtggcggatccgagctcgtgatgacccagactgcatcccccgtgtctgcagctgtgggaggcacagtcaccatcaattgccaggccagtcagagcattagcactgcattagcctggtatcagcagagaccagggcagcctccccgtctcctgatctacgatgcatccactctggcatctggggtctcatcgcggttctctggcagtggatctgggacagagttcactctcaccatcagcgacctggagagtgccgatgctgccacttactactgtcaaacctattttggtagtgatactgataatgctttcggcgaagggaccgaggtggagatcacaggttcggcggccgcaggtggaggcggttcaaaaaagaaaatcgag

SEQ ID NO: 12 - DNA, 780 bp, Artificial Sequence
  example
caggagcagctggtggagtccgggggaggcctggtcactcctggaggaaccctgacactcacctgcacagtctctggaatcgacctcagtagctatgcaatgagctgggtccgccaggttccaggggaagggctggaatggatcggaatcattggtagtggtggtggcacagcctacgcgaactgggcgcgtggccgattcaccatctcccgtacctcgtcgaccacggtggatctgcgtatgaccagtctgacaaccgaggacacggccacctatttctgtgccaccgattacggcatttatggttatgcttatggtcacttgtggggcccaggcaccctcgtcaccgtcactagtggtggaggcggttcaggcggaggtggctctggcggtggcggatccgagctcgtgatgacccagactgcatcccccgtgtctgcagctgtgggaggcacagtcaccatcaattgccaggccagtcagagcattagcactgcattagcctggtatcagcagagaccagggcagcctccccgtctcctgatctacgatgcatccactctggcatctggggtctcatcgcggttctctggcagtggatctgggacagagttcactctcaccatcagcgacctggagagtgccgatgctgccacttactactgtcaaacctattttggtagtgatactgataatgctttcggcgaagggaccgaggtggagatcacaggttcggcggccgcaggtggaggcggttcaaagaagaaaaagaaaatcgag

SEQ ID NO: 13 - protein, 8 aa, Artificial Sequence
  spacer
AAAGGGGS

SEQ ID NO: 14 - protein, 11 aa, Artificial Sequence
  spacer
AAAGGGGSKIE

SEQ ID NO: 15 - protein, 13 aa, Artificial Sequence
  spacer
AAAGGGGSKKKIE

SEQ ID NO: 16 - protein, 15 aa, Artificial Sequence
  spacer
AAAGGGGSKKKKKIE

SEQ ID NO: 17 - protein, 20 aa, Artificial Sequence
  spacer
GGGGSGGGGSGGGGSGGGGS

SEQ ID NO: 18 - protein, 121 aa, Oryctolagus cuniculus
QSVKESGGRLVTPGTPLTLTCTVSGIDLSSNAMSWVRQAPGEGLEWIGTISTVGKTYFASWAKGRFTISKTSTTVDLRITSPTTEDTATYFCATRYDSYGYAYNYWFGTLWGPGTLVTVTS

SEQ ID NO: 19 - protein, 117 aa, Oryctolagus cuniculus
QSVKESEGRLVTPGTPLTLTCTVSGFSLSRYAVSWVRQAPGKGLEWIGIIGSGGSTSYATWARGRFTISKTSTTVDLKITSPTTEDTVTYFCGSYYDSHGYAYVSLWGPGTLVTVTS

SEQ ID NO: 20 - protein, 118 aa, Oryctolagus cuniculus
QQQLMESGGRLVTPGGSLTLTCTVSGIDLNSYAMGWVRQAPGKGLEYIGIIRNSGNTYYASWAKGRFTISKTSSTTVDLKMTSLTTEDTATYFCARYSGDNGGALNLWGPGTLVTVTS

SEQ ID NO: 21 - protein, 121 aa, Oryctolagus cuniculus
QSLEESGGRLVTPGTPLTLTCTVSGIDLSSNAMTWVRQAPGEGLEWIGTISTGGSTYFASWAKGRFTISKTSTTVDLKITSPTTEDTATYFCATRYDSYGYAYNYWFGTLWGPGTLVTVTS

SEQ ID NO: 22 - protein, 116 aa, Oryctolagus cuniculus
QSVKESGGRLVTPGTPLTLTCTVSGFSLSSYAMGWVRQAPGKGLEYIGIISSSGSTYYASWAKGRFTISKTSTTVDLKITSPTTEDTATYFCARYSGDNGGALNLWGPGTLVTVTS

SEQ ID NO: 23 - protein, 116 aa, Oryctolagus cuniculus
QQQLMESGGGLVTPGTPLTLTCTVSGIDLRRYAMGWVRQAPGKGLQWIGIIASGNTDYASWAKGRFTISATSTTVDLKITSSTTEDTATYFCARYSGDNGGTLNLWGPGTLATVTT

SEQ ID NO: 24 - protein, 121 aa, Oryctolagus cuniculus; identical to SEQ ID NO: 21

SEQ ID NO: 25 - protein, 115 aa, Oryctolagus cuniculus
QSLEESGGRLVTPGTPLTLTCTVSGIDLRRYAMGWVRQAPGKGLQWIGIIASGNTDYASWAKGRFTISATSTTVDLKITSPTTEDTATYFCARYSGDNGGTLNLWGPGTLVTVTS

SEQ ID NO: 26 - protein, 112 aa, Oryctolagus cuniculus
ELDLTQTPPSVSGAVGGTVTIKCQASENINSELAWYQQKPGQRPKLLIYDASKLASGVPSRFSGSGSGTEYTLTISGMQCDDAATYYCQSTYYDGNYVYAFGGGTEVDVTRS

SEQ ID NO: 27 - protein, 111 aa, Oryctolagus cuniculus
ELVLTQTPSPVSGAVGGTVTINCQASQSISTALAWYQQKPGQPPKLLIYSASTLASGVSSRFKGSGSGTGFTLTISDLECADAATYYCFGGGTEVVIKRSQSYYGSSSDNA

SEQ ID NO: 28 - protein, 113 aa, Oryctolagus cuniculus
ELVMTQTAASVSGPVGGTVTIKCQASEFIRNYLAWYQQKPGQPPKLLIYTTSNLASGVPSRFSGSGSGTEYTLTISDLECADAATYYCQNYYDISTYGNAFGGGTEVVVIKGS

SEQ ID NO: 29 - protein, 112 aa, Oryctolagus cuniculus
ELVMTQTAASVSEPVGGTVTIKCQASQNINNELAWYQQKPGQRPKLLIYDASKLASGVPSRFSGSGSGTEFTLTISGMQCDDAATYYCQSTYYDGNYVYAFGGGTEVDVKGS

SEQ ID NO: 30 - protein, 112 aa, Oryctolagus cuniculus
ELDLTQTAASVSEPVGGTVTISCQSSQHIRSYLAWYQQKPGQPPKLLISAASTLASGVSSRFKGSGSGTEFTLTISDLECADAATYYCQRYYDIRNYGNGFGGGTEVEITGS

SEQ ID NO: 31 - protein, 112 aa, Oryctolagus cuniculus
ELVMTQTAASVSEPVGGTVTIKCQASEHIRNYLAWYQQKPGQPPKLLIYTTSNLASGVPSRFSGSGSGTEYTLTISDLECADAATYYCQNYYDISTYGNTFGGGTEVDVKGS

SEQ ID NO: 32 - protein, 112 aa, Oryctolagus cuniculus
ELVMTQTAASVSEPVGGTVTINCQASQSISDELAWYQQKPGQRPKLLIYDASDLASGVPSRFSGSGSGTEFTLTISGVQCDDAATYYCQSAYYDGRYVYAFGGGTEVEVTGS

SEQ ID NO: 33 - protein, 112 aa, Oryctolagus cuniculus
ELVMTQTAASVSEPVGGTVTIKCQASQSISSYLAWYQQKPGQPPKLLIYAASNLASGVSSRFKGSGSGTEFTLTISDLECADAATYYCQSYYSISSYGNTFGGGTEVEITGS